European Patent Application EP 4 407 038 A1, published July 31, 2024. Title: Method for Preparing Starch Using Carbon Dioxide, Recombinant Microorganism, and Method for Constructing Recombinant Microorganism. Applicant: Tianjin Institute of Industrial Biotechnology. Application EP. The sequence listing filed with the application follows.

SEQUENCE LISTING (30 sequences)

SEQ ID NO: 1 - protein, 477 aa, synthetic construct [sequence omitted]

SEQ ID NO: 2 - DNA, 1434 bp, synthetic construct
  source 1..1434: mol_type = other DNA
atgcaagttttgcatgtttgttctgaaatgtttccattgttgaaaacgggtggtttggcggacgtcattggtgctttgcctgctgctcaaattgctgatggggtggatgctagagttttgttgcctgcttttcctgatattagaagaggtgttactgatgctcaagttgtatcgagaagggatacttttgctggtcatattactttgttgtttggtcattataatggtgttggtatttatttgattgatgctccacatttgtatgatagacctggttctccatatcatgatactaatttgtttgcttatactgataatgttttgagatttgctttgctcggatgggttggtgctgaaatggcttctggtttggatccattttggagacctgatgttgttcatgctcatgattggcatgctggtttggctcctgcttatttggctgctagaggtagacctgctaaatctgtttttactgttcataatttggcttatcaaggtatgttttatgctcatcacatgaacgatatccaattgccatggtctttctttaacattcacggtttggaatttaacggtcagatttcttttttgaaagctggtttgtattatgctgatcatattactgctgtttctccaacttatgctagagaaattactgaaccacaatttgcttatggtatggaaggtttgttgcaacaaagacatagagaaggtagattgtctggcgttttgaatggtgttgatgagaaaatttggtctcctgaaactgatttgttgttggcttctagatatactagagatactttggaagataaagctgaaaataaaagacaattgcaaattgctatgggtttgaaagttgatgataaagttccattgtttgctgtcgtctctaggttaacttctcaaaaaggtttggatttggttttggaagctttgcctggtttgttggaacaaggtggtcaattggctttgttgggggctggtgatcctgttttgcaagaaggttttttggctgctgctgctgaatatcctggtcaagttggtgttcaaattggttatcatgaagctttttctcatagaattatgggtggtgcagacgttattttggtgccatctagatttgaaccatgtggtttgactcaattgtatggtttgaaatatggtactttgccattggttagaagaactggtggtttggctgacactgtttctgattgttctttggaaaatttggctgatggcgttgcgtctggttttgtttttgaagattctaatgcttggtctttgttgagagctattagaagagcttttgttttgtggtctaggccgtctttgtggagatttgttcaaagacaagctatggctatggatttttcttggcaagttgctgctaaatcttatagagaattgtattatagattgaaataa

SEQ ID NO: 3 - protein, 431 aa, synthetic construct
MVSLEKNDHLMLARQLPLKSVALILAGGRGTRLKDLTNKRAKPAVHFGGKFRIIDFALSNCINSGIRRMGVITQYQSHTLVQHIQRGWSFFNEEMNEFVDLLPAQQRMKGENWYRGTADAVTQNLDIIRRYKAEYVVILAGDHIYKQDYSRMLIDHVEKGARCTVACMPVPIEEASAFGVMAVDENDKIIEFVEKPANPPSMPNDPSKSLASMGIYVFDADYLYELLEEDDRDENSSHDFGKDLIPKITEAGLAYAHPFPLSCVQSDPDAEPYWRDVGTLEAYWKANLDLASVVPELDMYDRNWPIRTYNESLPPAKFVQDRSGSHGMTLNSLVSGGCVISGSVVVQSVLFSRVRVNSFCNIDSAVLLPEVWVGRSCRLRRCVIDRACVIPEGMVIGENAEEDARRFYRSEEGIVLVTREMLRKLGHKQER

SEQ ID NO: 4 - DNA, 1296 bp, synthetic construct
  source 1..1296: mol_type = other DNA
atggtttctttggaaaaaaatgatcatttgatgttggctagacaattgccattgaaatctgttgctttgatcttggctggtggtagaggtactagattgaaagatttgactaataaaagagctaaacctgctgtacattttggtggtaaatttagaataatagattttgctctgtctaactgcattaattctggtattagaagaatgggtgttattactcaatatcaatctcatactttggtgcaacatattcaaagaggatggtcattctttaatgaagaaatgaatgaatttgttgatttgttgcctgctcaacaaagaatgaaaggtgaaaattggtatagaggtactgctgatgctgttactcaaaatttggatattattagaagatataaagctgagtatgttgttatattggctggggatcatatttacaaacaagattattctagaatgttgattgatcatgttgaaaaaggtgctagatgtactgttgcttgtatgcctgttccaattgaagaagcttctgcttttggtgttatggctgttgatgaaaatgataaaattattgaatttgttgaaaaacctgctaatccaccatctatgccaaatgatccatctaaatctttggcttctatgggtatttatgtttttgatgctgattatttgtatgaattgttggaggaggatgatagagatgaaaactcatctcatgattttggtaaagatttgattccaaaaattactgaagctggtttggcttatgctcatccatttccattgtcttgtgttcaatctgatcctgatgctgaaccatattggagagatgttggtactttggaagcttattggaaagctaatttggatttggcttctgttgttgatgaattggatatgtatgatagaaattggccaattagaacttataatgaatctttgccacctgctaaatttgttcaagatagatctggttctcatggtatgactttaaattctttggtttctgatggttgtgttatttctggttctgtggttgtgcaaagtgttttgttttctagagttagagttaattctttttgtaatattgattctgctgttttgttgcctgaagtttgggttggtagatcttgtagattgagaagatgtgttattgatagagcttgtgttattcctgaaggtatggttattggtgaaaatgctgaagaagatgctagaagattttatagatctgaagaaggtattgttttggttactagagaaatgttgagaaaattgggtcataaacaagaaagataa

SEQ ID NO: 5 - RNA, 20 nt, synthetic construct
  source 1..20: mol_type = other RNA
gagtcgataacgatctcctt

SEQ ID NO: 6 - RNA, 20 nt, synthetic construct
  source 1..20: mol_type = other RNA
gttgttgatgtagccgtcta

SEQ ID NO: 7 - RNA, 20 nt, synthetic construct
  source 1..20: mol_type = other RNA
ggacgtgatcagggaacatg

SEQ ID NO: 8 - RNA, 20 nt, synthetic construct
  source 1..20: mol_type = other RNA
ggccacctccgactcaatca

SEQ ID NO: 9 - RNA, 20 nt, synthetic construct
  source 1..20: mol_type = other RNA
gttaataagagcgttgtcca

SEQ ID NO: 10 - RNA, 20 nt, synthetic construct
  source 1..20: mol_type = other RNA
gagaagtcaaactcggtggt

SEQ ID NO: 11 - DNA, 1434 bp, synthetic construct
  source 1..1434: mol_type = other DNA
atgcaggtcctgcacgtctgcagcgaaatgttcccgctgctgaagaccggcggcctggccgacgtgatcggcgccctgccggccgcccagatcgccgacggcgtggacgcccgcgtgctcctgccggcgttcccggatatccgccgcggcgttacggacgcccaggtggtctcgcgccgcgacaccttcgcgggtcacatcaccctgctgttcggtcactacaacggtgtgggtatctacctgatcgacgctccgcatctgtacgaccgcccgggctccccgtaccatgatacgaacctcttcgcctacaccgacaacgtgctgcgcttcgcgctgctgggttgggtgggcgccgaaatggcatccggcctggaccctttctggcggccggacgtggtgcacgcccacgactggcatgccggcctggcaccggcttacctggccgcccgcggccgccctgccaaatcggtcttcaccgtccacaacctggcgtaccaaggcatgttctacgcgcatcacatgaacgacatccagctgccgtggtcgttcttcaacatccacggcctggagttcaacggccaaatctcgttcctgaaggcgggcctgtattacgccgatcacatcaccgccgtgtccccgacctacgcgcgcgagatcaccgagccgcagttcgcgtacggcatggaaggcctgctgcaacagcgccaccgcgaaggccgcctgtccggcgtcctcaacggtgtggatgagaagatctggtcccccgagaccgacctgctgcttgccagccgttacacccgcgacaccctcgaggataaggccgaaaacaagcgccagctgcagatcgcaatgggcctgaaagtggacgacaaggtgccactgttcgccgtcgtctctcgcctgacgagccagaagggcctggacctggttctcgaagccctgccgggcctgctggaacaaggcggccagctggcgctgctgggcgccggcgacccggtcctgcaggagggcttcctcgcggccgccgccgaatatccgggccaggtcggcgtgcagatcggctaccacgaagcattctcccatcgcatcatgggcggcgctgacgtgatcctggtgccgagccgcttcgaaccgtgcggtctgacgcagctgtacggtctcaagtacggcacgctgccgctggtccgtcgtaccggcggcctggccgacacggtctcagattgcagcctggaaaacctcgccgacggcgtcgcgtcgggcttcgtcttcgaggattcgaacgcctggtcgctactgcgtgcgatccgccgggcgttcgtgctctggtcccgtccgagtctgtggcgcttcgtgcaacgccaagcgatggccatggacttctcgtggcaggtggccgccaagtcgtaccgcgaactgtactaccgcctgaagtaa

SEQ ID NO: 12 - DNA, 1296 bp, synthetic construct
  source 1..1296: mol_type = other DNA
atggtttcgctggagaagaacgaccacctgatgctcgcccgccagctgccgctcaagtcggtggccctgatcctggccggcggtcgtggcacccgtctgaaggatctgaccaacaagcgtgcaaagccggctgtgcatttcggcggtaagtttcgcatcatcgatttcgccctgtcgaactgcatcaactcgggcattcgccgtatgggcgtcatcacccagtaccagtcgcacactctggtccaacacatccagcgcggctggtcgttcttcaacgaggaaatgaacgagttcgtggatctgctgccggcccagcagcgcatgaagggcgaaaactggtaccgcggcaccgcagacgctgtgacccagaacctggacatcattcgtcgctacaaggccgagtatgtcgtcatcctggctggcgaccatatctacaagcaggactactcgcgcatgctgatcgatcacgtggagaagggcgcccgctgcaccgtcgcgtgcatgccggtgccgatcgaagaggcctccgccttcggcgtcatggcagtcgatgagaacgacaagatcatcgaatttgtcgaaaagccggcgaatccgccgtctatgccgaacgacccgtcgaagtcgctggcctcgatgggcatctacgtgttcgacgcagactacctgtacgaactcctggaagaagacgaccgtgacgagaacagctcgcacgacttcggtaaggacctgatcccgaagatcaccgaagccggcctggcctacgcgcacccgttcccgctgagctgcgtgcagtccgacccggacgccgagccgtactggcgcgacgtgggcacgctcgaggcgtactggaaggccaacctggacctggcttcggtcgtcccggaactggacatgtacgaccgcaactggccgatccgtacctacaacgaatcgctgcccccggccaagttcgtgcaggaccgctcgggctcccacggtatgacgctgaactcgctggtgtcgggtggctgcgtcatttcgggctcggtcgtggtccagagcgtcctgttctcgcgcgtgcgcgtcaatagcttctgcaacatcgactcggcagttctgctgccggaggtttgggtgggccgctcgtgccgcctccgtcgctgcgtgatcgatcgcgcctgcgtcatccccgagggtatggtaatcggcgagaacgccgaggaggacgcccgccgtttctaccgctcggaagaaggtattgtgctcgtcacccgtgaaatgctgcgcaagttgggacacaagcaggaacgttaa

SEQ ID NO: 13 - protein, 423 aa, synthetic construct
MKAQPPLRLTAQAMAFVLAGGRGSRLKELTDRRAKPAVYFGGKARIIDFALSNAMNSGIRKMAIATQYKAHSLIRHIQRGWNFFREERNEYLDILPASQRVDENRWYLGTADAVTQNIDIVDSYDIKYVIILAGDHVYKMDYEIMLRQHCETGADVTIGCLTVPRAEATAFGVMHVDANLRITDFLEKPADPPGIPGDEANALASMGIYVFDWAFLRDLLIRDAEDPNSSHDFGHDLIPAIVKNGKAMAHRFSDSCVMTGLETEPYWRDVGTIDAFWQANIDLTDFTPKLDLYDREWPIWTYSQIVPPAKFIHDSENRRGTAISSLVSGDCIVSGSEIRSSLLFTGCRTHSYSSMSHVVALPHVTVNRKADLTNCVLDRGVVVPEGLVIGQDAEEDARWFRRSEGGIVLVTQDMLDARARALN

SEQ ID NO: 14 - protein, 431 aa, synthetic construct; identical to SEQ ID NO: 3

SEQ ID NO: 15 - protein, 431 aa, synthetic construct
MVSLEKNDRLMLARQLPLKSVALILAGGRGTRLKDLTNKRAKPAVHFGGKFRIIDFALSNCLNSGIRRIGVITQYQSHTLVQHIQRGWSLFSEEMNEFVDLLPAQQRMQGENWYRGTADAVTQNLDIIRRYKAEYVVILAGDHIYKQDYSRMLIDHVEKGARCTVACMPVPIKEATAFGVMAVDESEKIIDFVEKPANPPAMPGDDSKALASMGIYVFDADYLYELLAADDKDDASSHDFGKDIIPKITREGMAYAHPFPLSCVQSDPDAEPYWRDVGTLEAYWKANLDLASVTPELDMYDQNWPIRTHMESLPPAKFVQDRSGSHGMTLNSLVSGGCIISGSVVVQSVLFPRVRINSFCNIDSAVLLPEVWVGRSCRLRRCIIDRACIIPEGMVIGENAEEDARRFYRSEEGIVLVTREMLRKLQVKQER

SEQ ID NO: 16 - protein, 476 aa, synthetic construct
MVRFESTDSLMLARQLPNKTVALILAGGRGSRLKDLTATRAKPAVHFGGKFRIIDFALSNCLNSGVRRIGVITQYQSHTLVQHIQRGWSFLNEEMNEFVDLLPAQQRLSTEQWYKGTADAVCQNLDIIRRYDAEYIVILAGDHIYKMDYSRMLLDHVEKGAECTVACIPVPISEGSEFGIMEVTADYQITAFYEKPANPPPIPGDPSNALASMGIYIFNADYLFKLLEEDNNTPGSSHDFGKDIIPQLTARKVVWAHPFDLSCVTSNAELPPYWRDVGTLDAYWRANLDLASVTPELDMYDRAWPIRTHMEPLPPAKFVQDRSGSHGMTMNSLVSGGCIVSGSVVVHSVLFPRVRVNSFCTIDSSLLLPDVHVGRSCRLRRCIIDRACHIPEGMVIGENADEDNARFYRSEGGGGVSDSGYAGKVRGKIEPLGFLFVRLDLLIRLSLLIRLNLFIRMNLLIILTLFFKLASIQASH

SEQ ID NO: 17 - protein, 420 aa, synthetic construct
MRKVLALILAGGHGKRLGVLTEKIAKPAVPFGGKYRLIDFTLSNCVNSGIYHVGVLTQYRPHLLNNHINIGRPWDLDRKKGGVTILPPYLGGVAGWYRGTANAVYQNIEYVDSADPDFVLILSGDHVYAMDYNDIIDFHILKGAEGTIACIEVPPEETNRFGIMMTDLDSRIVDFEEKPQRARSNLASLGIYVFNWKFLKEYLIRDEQNNESTHDFGHDIIPLMINEGCQIYAFKFNGYWRDVGTVRSYWESNLELTRPIPPLNLYDRHWRFFTQTEEMPPAYCAPTSKIVNSIISEGCEIYGFVENSVIFQGVYIGENAVVKNSVVMTSTKIGENCVITDAVIAERVIVENRVIIGEGDDAKNKLDSDVYTGQITVIGMYSVIPSGSVIGKNCVVGVGVEKGDFKTQKVESGDYILHKE

SEQ ID NO: 18 - protein, 376 aa, synthetic construct
MAQKQKCVAMLLAGGKGSRLSALTKNLAKPAVPFGGKYRIIDFTLSNCANSGIETVGILTQYQPLELHNYIGIGNAWDLDRVSGGVTVLPPYAESSGVKWYTGTASAIYQNLNYLSQYEPEYVLILSGDHIYKMDYSKMLDYHIEKEADVSISVIEVPWDEASRFGIMNTNEEMEIVEFEEKPQFPRSNLASMGIYIFNWAILKEYLEMDARNPESSNDFGKDVLPLLLDEGKKLMAYPFEGYWKDVGTVKSLWEANMDLLRDETSLNLNDRDWRIYSVNPNEPPQYIAEKARVEESLINEGCVIEGDVKHSVLFQGVTVEEGSMVIDSVVMPGAKIGKNVVIERAIVGSEMVIEDGTIIRPEKNVDDVVLIAEGK

SEQ ID NO: 19 - protein, 404 aa, synthetic construct
MREVPHVLGIVLAGGEGKRLYPLTADRAKPAVPFGGAYRLIDFVLSNLVNARYLRICVLTQYKSHSLDRHISQNWRLSGLAGEYITPVPAQQRLGPRWYTGSADAIYQSLNLIYDEDPDYIVVFGADHVYRMDPEQMVRFHIDSGAGATVAGIRVPRENATAFGCIDADDSGRIRSFVEKPLEPPGTPDDPDTTFVSMGNYIFTTKVLIDAIRADADDDHSDHDMGGDIVPRLVADGMAAVYDFSDNEVPGATDRDRAYWRDVGTLDAFYDAHMDLVSVHPVFNLYNKRWPIRGESENLAPAKFVNGGSAQESVVGAGSIISAASVRNSVLSSNVVVDDGAIVEGSVIMPGTRVGRGAVVRHAILDKNVVVGPGEMVGVDLEKDRERFAISAGGVVAVGKGVWI

SEQ ID NO: 20 - protein, 420 aa, synthetic construct
MSNVRYISNLTRETYALILAGGRGSRLHELTDWRAKPALYFGGKFRIIDFPLSNCINSGIRRVGVVTQYKSHSLIRHVMRGWGHFKKELGESVEILPASQRYSENWYQGTADAVFQNIDIIRHELPKYVMVLSGDHVYRMDYAGLLAAHAESGADMTVSCLEVPVAEAAGAFGVMEVDDDMRILGFEEKPQLPKHCPGNPEKCLASMGNYVFNTEFLFEQLKKDAQNAESDRDFGKDIIPSIIEKHKVFAYPFKSAFPNEQAYWRDVGTLDSFWLANMELLSPTPALNLYDAKWPIWTYQEQLPPAKFVFDDDDRRGMAVDSIISGGCIISGATVRRSVLFNEVRVCSYSVVEDSVVLPDVVVLRHCKIKNAIIDRGCIIPEGTVIGYNHDHDRAKGFRVSEKGITLVTRDMLGLPVGYE

SEQ ID NO: 21 - protein, 431 aa, synthetic construct; identical to SEQ ID NO: 3

SEQ ID NO: 22 - protein, 478 aa, synthetic construct
METARGRVLSVASECVPLLKTGGLADVVGALPGALAAEGWEMRVLMPCYRPLKWRLEEMEEVFAEEDLFGGPGRVMAGEVAGRKMLLLDAPHLYDREGGPYAGPDGDWGDNAQRFAALSWIGARIAREGLGDGWRPDVVHAHDWQAGFTPAYMNYWGSGGASSVLTVHNIAFQGWAPASLLSALRLPPQEFHPAALEYYGGLSSLKAGLVSADHITTVSPTYACELMRPEFGMGLQGVIAQRAGQVTGILNGVDTDIWSPEVEERPYDAESLKAKAENRAVLSGAFKLSVPGPLAILVSRLTYQKGIDLIPEVLPDFIAAGGGLAVLGTGDAPLEAAMRELEVRFPGRVGVRIGYDEGLSHLMFAGGDAVLVPSRFEPCGLTQMYGLRYGAIPVVALTGGLADTIINANPAAMAAGCATGLTFHPTEPPAFAEALRRLIHLYADPAAWETVQRNAMRHPVGWETSAAAYAALYRELVA

SEQ ID NO: 23 - protein, 477 aa, synthetic construct [sequence omitted]

SEQ ID NO: 24 - protein, 878 aa, synthetic construct
MIFGTPNSTFLENRLGSSTGMPFSSATSLNSGVDQMMNELNIQQPTSHTVLFDLSWEVAKKVGGIYTVLKTKAPVTVEEYKSRYALIGPYNASTAPTEFEPLIPGPLSSPIIENMMKKYGIHVHFGKWLVEGYPKVFLIDLHSSMHKLGEWRWDLMSGFEQAGDNETNETIVFGYQSALLLKEFAEANPNDKYIAHFHEWQASVGLILLKKWKVPVSTIFTTHATLLGRYLAAGGVDLYNQMQVLNMDFEASKRGIYHRHWIEKKSAADSHVFTTVSEITGYESEHILMRKPDVILPNGLKLDKFTALHEFQNLHAKYKGVLNEFVRGHFYGHYSDFDLDNTLYVFTAGRHEYFNKGVDMFLDSLAGLNKLLQQSGSKMTVVAFIIMPAATNNFNVESLKGHSYLKDMRRTCNTIVEAMGERLFEATSRGKMISPEELLSQEDLVMLKRRIFALKQKSSGPPVVTHNMINDNDEILQHIRRIKLFNSQEDRVKVIYHPEFLTSTNPLIPLDYTEFVRGCHLGIFPSYYEPFGMTPAECCASGCPSITSNLTGFANYMSRALQDTDSKGIFIVDRRFKSSRETVDQMTQYLWKFTQLDRRQRIELRNATEKLSELLDWRTLGKFYKTARALALERAFPPKPISRSPSPSPSSSLKLSTGLSNQIELQQQQQQQQPQPIGTTINLIPPSSNVSVTPTTTPTTTTTATTATTAPITTPKPNVIPINTGKENITLLSPNSMSSLLSDSLNEFKKQQQQQQQSKTPTTPTTTSTTTTTPSTTAAATNKSVLSNPTPTPSPNTSSFIPTNKGSTATTTTTTATPTPTPSNNTNGKPFNPIEALTKSNSSSNFATTSTASVNTNNGGTNSPVSKSIPIPSSKSLK

SEQ ID NO: 25 - protein, 475 aa, synthetic construct
MKILFVSYEVYPLAKVGGLADVAGSLPKYLEKEGVSVQIAMPFHKKVKADNIENTGIVITTKHLPEKYSFEIYKTPLPGSGVPVFLFKNDQLIDSDEVYEGTDLALQAIAFSDAVVKFAETLEPDLLHVNDWQPALIPAYISAFYNGKPKTLLTIHNLGYQGEFDKSYFYKTGLPEKLWQEGKAVKNGAFNFLKTGIVTATAISTVSPTYAKEIQTPEYGAGLDETLRALSDRLFGILNGIDYSEYNPATDKRIPVNFDINSLEKKKENKIALQKELGLPVIDVPVIGLISRLVEQKGFDLIEAAAEKILSNDLQFVVLGTGEERYERLFKSLGERFPEKVSANITFNVDLAQKIYAGSDMFLMPSRYEPCGLGQMFAMRYGTIPVVRFTGGLRDTVKEFNPETLEGNGFGFEEYNPDKLLEAVEKAIKIYENKTLWNQLMLNAMNTDCSWDKSAREYIKLYKHVLNSGRDILNA

SEQ ID NO: 26 - protein, 476 aa, synthetic construct
MKILFVAAEGAPFAKTGGLGDVIGALPKSLVKNNNEVSVILPYYDVVDAKFGDQIEDLFYFFTNVGWRREYVGIKHIFRDGVDFYFIDNKHYFYRGQIYGEFDDGERFAYFQLAALEAMEKIQFIPDILHVHDYHTAMIPYLLKEKYHWINAYHGIKTVFTIHNIEFQGQFNPSMLGELFGVGDERYRDGTLRWNDCLNWMKAAVLYADRVTTVSPSYAKEIMTPEFGKGLDQIMRMESGKLSGVVNGIDTDLFDPETDPHLAVHFSKDDLSGKAKNKAALQERVGLPVREDVPLVGIVSRLTDQKGFQLVVDQLNTMMQLDLQIVLLGTGYADFENAFAWFGHAYPDKMSANITFDLELAQQIYAASDIFLMPSAFEPCGLSQMMAMRYGTLPLVHEVGGLRDTVIPYNEFEKTGTGFGFQDFSGYWLTKTLEAALDVYYNRKEDWKILQKNAMTTDFSWDTASQSYEHLYKELA

SEQ ID NO: 27 - protein, 476 aa, synthetic construct
MRVLHVCSELFPLLKTGGLADVIGALPAAQLAEGADVRIILPAFPDLRRGIPETVLVREIDTFAGRVALRYGHYRGIGIYLIDAPALYDRAGSPYHDASLYAYSDNYLRFALLGWMACELACGLDGYWRPEVVHAHDWHAGLTCAYLAARGRPARSVFTVHNLAYQGLFSADHLSELHLPAEFFQIYGLEFYGQISYLKAGLFFADHVTTVSPTYAKEITQPAFGYGMEGLLQALARQGRLTGILNGVDSDIWDPQSDTLLPTRYDAENLQAKAINKTHLQTAMGLQLAENKPIFAVVSRLTVQKGLDLVLEALPELLALGGQLVVLGSGDATLQEAFLAAAAEHSGQVGVQIGYHEAFSHRIIAGSDVILVPSRFEPCGLTQLYGLKYGTLPLVRHTGGLADTVVDCALENLADGSASGFVFNECEAQALVKAIRRAFVLWSRPKHWRHVQRHAMRLDFGWQLAAVDYLSLYRRL

SEQ ID NO: 28 - protein, 446 aa, synthetic construct
MRVLHVTSEVFPFSRSGGLGDVLGALPAVQATLGAQVSVLSPWYGSLAGAPEQIWAGDVADVGPVRVGELRQDGVRFLFLGLPEFEREGLYHPDDVWRFCTYGRAVLPVLRALNEVPDVLHGHDWQAGLVVAHAHEAGWRTVYTVHNLQYQGRWNLAEASGWSGLGPAWLTHEGAEFYGDLNLMKAGLIAANHVTTVSPQYAREITTQQYGEGLQGVLLRLTLEGRLSGIINGLDQERWNPRTDPDVPAYSDLAGKAAATQALRTEFGLDKAPVLGVVSRLADQKGMDLLIEALPRLVHNWNVVVLGGGDPLLTAALEGWAQHPRVSFAQGMNEALAHQIYAGSDAFAMPSRFEPCGLSQMIAMRYGTLPVVRETGGLVDTVPPDVGFRFQPATPEALVEACQQARAAFEDQSDWEARVARAMALDFSWDGPAREYLALYERVVTG

SEQ ID NO: 29 - protein, 508 aa, synthetic construct
MATKKTSLTKHPLKILFVSSEVEGFAKTGGLADVAKSLPAALKKMGHDVRIVMPFYQTINGKDNAVAILSTELLVESQPFAVSYQVMQLDEGNVPVYALDAPQYYDRPELYAENNQAYADNGERFTFLSAASLDLCEKLGFQPDVIHCNDWHTGLIPFLLKTRYAESDFFAKSKSVITIHNAVFKGVFNYDQYSLIPELIQRRYINAEMDPSHISMLKAGVAYADKVNAVSPNYASELLTHLGSHGMEADFQNRAKDLYGIINGCDYDDWNPETDVYIKQKFKANKVSLARGKKACRRDLQKQVNLPEVDVPVYGMVCRLTEQKGLHYLIPVLEDFLLNDVQVVIVGTGDPTLASALRDISEQHSDKFAFVETYSNPLAHCVEAGVDFFMMPSEFEPCGLNQMYSLAYGTLPIVRSVGGLKDTVIDYDQTPQVATGFIYDTPTPEALLIKLQRSLLLYCQRPQEFKRLQQNAMACKFNWDESAEQYLDMYLGGEQSLVNEICNDKVDA

SEQ ID NO: 30 - protein, 482 aa, synthetic construct
MNIVLAASEAFPFCKTGGLADVTGSLAKELSKHKGNRVILFLPHYRNINRVASLKVVPGTFLIPIGDRLETASLSYISWGNVLVFFINNTKYFDRPELYRTAAGDYFDNDERFIFFNRAVLESCKFIGYRPDIIHAHDWQAGLLPAYLKTVYKTDAFFTRTRSLFTIHNMAYQGQYPYSTFIKTGFHTVDYVPERFEYYGGISYLKSGIVYADYVNTVSPNYAKEITLDEKMGFGMEGLLRSRQDTFCGILNGLDTGVWDPEHDPLIPYSYESFSPVKGKAACKQFLQNMLGLEVSPSKPLVGIVSRMDYQKGLDLIPGVVNKYKDKVQFVVVGTGDSGMEKAFMALAKNNVGKVAYVAKVDEELAHRVYAGSDIFLMPSRFEPCGLSQMISMRYGTVPIVSRVGGLLDTVKGYDGITKYATGFFILEFSETGIERSLDYALKYYQDKRCWGMLIKNGMEKDFSWTKSAQEYQDLYKKIISK